European Patent Application EP 4 729 546 A1, published April 22, 2026. Title: ANTIBODIES SPECIFICALLY RECOGNIZING FACTOR XIIa AND USES THEREOF. Applicant: STAIDSON (BEIJING) BIOPHARMACEUTICALS CO., LTD. Application CN. The sequence listing filed with the application follows.

SEQUENCE LISTING (161 sequences)

SEQ ID NO: 1 - protein, 5 aa, synthetic construct
SQTMS

SEQ ID NO: 2 - protein, 5 aa, synthetic construct
GYHIH

SEQ ID NO: 3 - protein, 5 aa, synthetic construct
DYSMN

SEQ ID NO: 4 - protein, 7 aa, synthetic construct
SSSYYWV

SEQ ID NO: 5 - protein, 5 aa, synthetic construct
HYWMH

SEQ ID NO: 6 - protein, 7 aa, synthetic construct
SNSADWN

SEQ ID NO: 7 - protein, 5 aa, synthetic construct
SNWIG

SEQ ID NO: 8 - protein, 5 aa, synthetic construct
TNYMT

SEQ ID NO: 9 - protein, 5 aa, synthetic construct
SYWMH

SEQ ID NO: 10 - protein, 17 aa, synthetic construct
SISVISGRTYYADSVKG

SEQ ID NO: 11 - protein, 17 aa, synthetic construct
SISVISRRTYYADSVKG

SEQ ID NO: 12 - protein, 17 aa, synthetic construct
SISHISGRTYYADSVKG

SEQ ID NO: 13 - protein, 17 aa, synthetic construct
SISYISGRTYYADSVKG

SEQ ID NO: 14 - protein, 17 aa, synthetic construct
SSHVISGRTYYADSVKG

SEQ ID NO: 15 - protein, 17 aa, synthetic construct
SISVISGRYYYADSVKG

SEQ ID NO: 16 - protein, 17 aa, synthetic construct
SISVISGRAYYADSVKG

SEQ ID NO: 17 - protein, 17 aa, synthetic construct
SISVISGRKYYADSVKG

SEQ ID NO: 18 - protein, 17 aa, synthetic construct
SISVISGRPYYADSVKG

SEQ ID NO: 19 - protein, 17 aa, synthetic construct
SISVISGRSYYADSVKG

SEQ ID NO: 20 - protein, 17 aa, synthetic construct
SISVISKRTYYADSVKG

SEQ ID NO: 21 - protein, 17 aa, synthetic construct
SISVISGRNYYADSVKG

SEQ ID NO: 22 - protein, 17 aa, synthetic construct
SISVISGRDYYADSVKG

SEQ ID NO: 23 - protein, 17 aa, synthetic construct
SISVISGRRYYADSVKG

SEQ ID NO: 24 - protein, 17 aa, synthetic construct
SISVISGRMYYADSVKG

SEQ ID NO: 25 - protein, 17 aa, synthetic construct
SSSVISGRTYYADSVKG

SEQ ID NO: 26 - protein, 17 aa, synthetic construct
WIRVNGGNTMYARKFQG

SEQ ID NO: 27 - protein, 19 aa, synthetic construct
YISNSRSRSSKYYADSVKG

SEQ ID NO: 28 - protein, 16 aa, synthetic construct
SIYHSGSTYYNPSLKS

SEQ ID NO: 29 - protein, 17 aa, synthetic construct
GITSSGGSKYYADSVKG

SEQ ID NO: 30 - protein, 18 aa, synthetic construct
RTYYRSKWYNDYAVSVKS

SEQ ID NO: 31 - protein, 17 aa, synthetic construct
IIYPDDSDTRYSPSFQG

SEQ ID NO: 32 - protein, 16 aa, synthetic construct
VIYSGGSTYYADSVKG

SEQ ID NO: 33 - protein, 17 aa, synthetic construct
RINLDGSSTGYADSVRG

SEQ ID NO: 34 - protein, 6 aa, synthetic construct
SHAFDV

SEQ ID NO: 35 - protein, 6 aa, synthetic construct
AHAFDV

SEQ ID NO: 36 - protein, 6 aa, synthetic construct
SHAFDL

SEQ ID NO: 37 - protein, 6 aa, synthetic construct
WHAFDV

SEQ ID NO: 38 - protein, 6 aa, synthetic construct
SHRFDV

SEQ ID NO: 39 - protein, 6 aa, synthetic construct
GHAFDV

SEQ ID NO: 40 - protein, 6 aa, synthetic construct
HHAFDV

SEQ ID NO: 41 - protein, 6 aa, synthetic construct
QHAFDV

SEQ ID NO: 42 - protein, 6 aa, synthetic construct
SHDFDV

SEQ ID NO: 43 - protein, 12 aa, synthetic construct
RPYCSGGTCSDS

SEQ ID NO: 44 - protein, 15 aa, synthetic construct
IGYCKNGVCGGAYDY

SEQ ID NO: 45 - protein, 15 aa, synthetic construct
AATSGWYLRYWYFDL

SEQ ID NO: 46 - protein, 8 aa, synthetic construct
RGPPTHDS

SEQ ID NO: 47 - protein, 8 aa, synthetic construct
GGPRPLDI

SEQ ID NO: 48 - protein, 14 aa, synthetic construct
QGSSTYYRVGWFDP

SEQ ID NO: 49 - protein, 17 aa, synthetic construct
GRYYDGVDYGPKYGMDV

SEQ ID NO: 50 - protein, 7 aa, synthetic construct
SSRGFDP

SEQ ID NO: 51 - protein, 11 aa, synthetic construct
RASQSVYSNLA

SEQ ID NO: 52 - protein, 11 aa, synthetic construct
RASQSVYSALA

SEQ ID NO: 53 - protein, 11 aa, synthetic construct
RASQSVWSNLA

SEQ ID NO: 54 - protein, 11 aa, synthetic construct
RASQSVYYNLA

SEQ ID NO: 55 - protein, 11 aa, synthetic construct
RASQSLYSHLA

SEQ ID NO: 56 - protein, 11 aa, synthetic construct
RASQSVFSNLA

SEQ ID NO: 57 - protein, 11 aa, synthetic construct
RASESVFSNLA

SEQ ID NO: 58 - protein, 11 aa, synthetic construct
RASQAIRNNLA

SEQ ID NO: 59 - protein, 11 aa, synthetic construct
RANQNINSYLN

SEQ ID NO: 60 - protein, 11 aa, synthetic construct
QASQDITKYLN

SEQ ID NO: 61 - protein, 17 aa, synthetic construct
KSSQSVLYRSKRKPNLA

SEQ ID NO: 62 - protein, 11 aa, synthetic construct
RASQSISSYLN

SEQ ID NO: 63 - protein, 11 aa, synthetic construct
RASQSVRYNLA

SEQ ID NO: 64 - protein, 12 aa, synthetic construct
RASQSISSSYLA

SEQ ID NO: 65 - protein, 7 aa, synthetic construct
GASTRAT

SEQ ID NO: 66 - protein, 7 aa, synthetic construct
DGNKRAT

SEQ ID NO: 67 - protein, 7 aa, synthetic construct
TASSLES

SEQ ID NO: 68 - protein, 7 aa, synthetic construct
AATRLQS

SEQ ID NO: 69 - protein, 7 aa, synthetic construct
DASILET

SEQ ID NO: 70 - protein, 7 aa, synthetic construct
WASTRES

SEQ ID NO: 71 - protein, 7 aa, synthetic construct
AASSLQS

SEQ ID NO: 72 - protein, 7 aa, synthetic construct
GASIRAT

SEQ ID NO: 73 - protein, 7 aa, synthetic construct
GASRRAT

SEQ ID NO: 74 - protein, 9 aa, synthetic construct
QQYNKWPLS

SEQ ID NO: 75 - protein, 9 aa, synthetic construct
QQYHKWPLS

SEQ ID NO: 76 - protein, 9 aa, synthetic construct
QQNNKWPLS

SEQ ID NO: 77 - protein, 9 aa, synthetic construct
QQYKKWPLS

SEQ ID NO: 78 - protein, 9 aa, synthetic construct
QQYHWWPLS

SEQ ID NO: 79 - protein, 9 aa, synthetic construct
QQNNRWPLS

SEQ ID NO: 80 - protein, 9 aa, synthetic construct
QQYQKWPLS

SEQ ID NO: 81 - protein, 10 aa, synthetic construct
HQYNNWPPET

SEQ ID NO: 82 - protein, 9 aa, synthetic construct
LQYHDSPWT

SEQ ID NO: 83 - protein, 9 aa, synthetic construct
QQSYSSLRT

SEQ ID NO: 84 - protein, 9 aa, synthetic construct
QHYNSYSWT

SEQ ID NO: 85 - protein, 9 aa, synthetic construct
QQYYSTPLT

SEQ ID NO: 86 - protein, 9 aa, synthetic construct
QQSYSTPQT

SEQ ID NO: 87 - protein, 9 aa, synthetic construct
QFYGSSPLT

SEQ ID NO: 88 - protein, 9 aa, synthetic construct
QLYGHSAYT

SEQ ID NO: 89 - protein, 17 aa, synthetic construct
  VARIANT 2: note = X is I or S
  VARIANT 3: note = X is H or S
  VARIANT 4: note = X is H, V or Y
  VARIANT 7: note = X is G, K or R
  VARIANT 9: note = X is A, D, K, M, N, P, R, S, T or Y
SXXXISXRXYYADSVKG

SEQ ID NO: 90 - skipped

SEQ ID NO: 91 - protein, 11 aa, synthetic construct
  VARIANT 6: note = X is L or V
  VARIANT 7: note = X is F, W or Y
  VARIANT 8: note = X is S or Y
  VARIANT 9: note = X is A, H or N
RASQSXXXXLA

SEQ ID NO: 92 - protein, 9 aa, synthetic construct
  VARIANT 3: note = X is N or Y
  VARIANT 4: note = X is H, K, N or Q
  VARIANT 5: note = X is K, R or W
QQXXXWPLS

SEQ ID NO: 93 - protein, 115 aa, synthetic construct
EVQLLESGGGLVQPGGSLRLSCAGSGFSFGSQTMSWVRQAPGKGLEWVSSISVISGRTYYADSVKGRFTISRDNSKNTLYLQMNSLRAEDTAVYYCTKSHAFDVWGQGTMVTVSS

SEQ ID NO: 94 - protein, 115 aa, synthetic construct
EVQLLESGGGLVQPGGSLRLSCAGSGFSFGSQTMSWVRQAPGKGLEWVSSISVISRRTYYADSVKGRFTISRDNSKNTLYLQMNSLRAEDTAVYYCTKSHAFDVWGQGTMVTVSS

SEQ ID NO: 95 - protein, 115 aa, synthetic construct
EVQLLESGGGLVQPGGSLRLSCAGSGFSFGSQTMSWVRQAPGKGLEWVSSISHISGRTYYADSVKGRFTISRDNSKNTLYLQMNSLRAEDTAVYYCTKSHAFDVWGQGTMVTVSS

SEQ ID NO: 96 - protein, 115 aa, synthetic construct
EVQLLESGGGLVQPGGSLRLSCAGSGFSFGSQTMSWVRQAPGKGLEWVSSISYISGRTYYADSVKGRFTISRDNSKNTLYLQMNSLRAEDTAVYYCTKSHAFDVWGQGTMVTVSS

SEQ ID NO: 97 - protein, 115 aa, synthetic construct
EVQLLESGGGLVQPGGSLRLSCAGSGFSFGSQTMSWVRQAPGKGLEWVSSSHVISGRTYYADSVKGRFTISRDNSKNTLYLQMNSLRAEDTAVYYCTKSHAFDVWGQGTMVTVSS

SEQ ID NO: 98 - protein, 115 aa, synthetic construct
EVQLLESGGGLVQPGGSLRLSCAGSGFSFGSQTMSWVRQAPGKGLEWVSSISVISGRYYYADSVKGRFTISRDNSKNTLYLQMNSLRAEDTAVYYCTKSHAFDVWGQGTMVTVSS

SEQ ID NO: 99 - protein, 115 aa, synthetic construct
EVQLLESGGGLVQPGGSLRLSCAGSGFSFGSQTMSWVRQAPGKGLEWVSSISVISGRAYYADSVKGRFTISRDNSKNTLYLQMNSLRAEDTAVYYCTKSHAFDVWGQGTMVTVSS

SEQ ID NO: 100 - protein, 115 aa, synthetic construct
EVQLLESGGGLVQPGGSLRLSCAGSGFSFGSQTMSWVRQAPGKGLEWVSSISVISGRKYYADSVKGRFTISRDNSKNTLYLQMNSLRAEDTAVYYCAKSHAFDVWGQGTMVTVSS

SEQ ID NO: 101 - protein, 115 aa, synthetic construct
EVQLLESGGGLVQPGGSLRLSCAGSGFSFGSQTMSWVRQAPGKGLEWVSSISVISGRAYYADSVKGRFTISRDNSKNTLYLQMNSLRAEDTAVYYCTKAHAFDVWGQGTMVTVSS

SEQ ID NO: 102 - protein, 115 aa, synthetic construct
EVQLLESGGGLVQPGGSLRLSCAGSGFSFGSQTMSWVRQAPGKGLEWVSSISYISGRTYYADSVKGRFTISRDNSNNTLYLQMNSLRAEEPAVYYCTKSHAFDLWGRGTMATWSP

SEQ ID NO: 103 - protein, 115 aa, synthetic construct
EVQLLESGGGLVQPGGSLRLSCAGSGFSFGSQTMSWVRQAPGKGLEWVSSISVISGRTYYADSVKGRFTISRDNSKNTLYLQMNSLRAEDTAVYYCTKWHAFDVWGQGTMVTVSS

SEQ ID NO: 104 - protein, 115 aa, synthetic construct
EVQLLESGGGLVQPGGSLRLSCAGSGFSFGSQTMSWVRQAPGKGLEWVSSISVISRRTYYADSVKGRFTISRDNSKNTLYLQMNSLRAEDTAVYYCTRSHAFDVWGQGTMVTVSS

SEQ ID NO: 105 - protein, 115 aa, synthetic construct
EVQLLESGGGLVQPGGSLRLSCAGSGFSFGSQTMSWVRQAPGKGLEWVSSISHISGRTYYADSVKGRFTISRDNSKNTLYLQMNSLRAEDTAVYYCTKSHRFDVWGQGTMVTVSS

SEQ ID NO: 106 - protein, 115 aa, synthetic construct
EVQLLESGGGLVQPGGSLRLSCAGSGFSFGSQTMSWVRQAPGKGLEWVSSISVISGRPYYADSVKGRFTISRDNSKNTLYLQMNSLRAEDTAVYYCTKSHAFDVWGQGTMVTVSS

SEQ ID NO: 107 - protein, 115 aa, synthetic construct
EVQLLESGGGLVQPGGSLRLSCAGSGFSFGSQTMSWVRQAPGKGLEWVSSISVISGRSYYADSVKGRFTISRDNSKNTLYLQMNSLRAEDTAVYYCAKSHAFDVWGQGTMVTVSS

SEQ ID NO: 108 - protein, 115 aa, synthetic construct
EVQLLESGGGLVQPGGSLRLSCAGSGFSFGSQTMSWVRQAPGKGLEWVSSISYISGRTYYADSVKGRFTISRDNSKNTLYLQMNSLRAEDTAVYYCTKGHAFDVWGQGTMVTVSS

SEQ ID NO: 109 - protein, 115 aa, synthetic construct
EVQLLESGGGLVQPGGSLRLSCAGSGFSFGSQTMSWVRQAPGKGLEWVSSISVISGRSYYADSVKGRFTISRDNSKNTLYLQMNSLRAEDTAVYYCTKHHAFDVWGQGTMVTVSS

SEQ ID NO: 110 - protein, 115 aa, synthetic construct
EVQLLESGGGLVQPGGSLRLSCAGSGFSFGSQTMSWVRQAPGKGLEWVSSISVISKRTYYADSVKGRFTISRDNSKNTLYLQMNSLRAEDTAVYYCTRSHAFDVWGQGTMVTVSS

SEQ ID NO: 111 - protein, 115 aa, synthetic construct
EVQLLESGGGLVQPGGSLRLSCAGSGFSFGSQTMSWVRQAPGKGLEWVSSISVISGRSYYADSVKGRFTISRDNSKNTLYLQMNSLRAEDTAVYYCTKSHAFDVWGQGTMVTVSS

SEQ ID NO: 112 - protein, 115 aa, synthetic construct
EVQLLESGGGLVQPGGSLRLSCAGSGFSFGSQTMSWVRQAPGKGLEWVSSISHISGRTYYADSVKGRFTISRDNSKNTLYLQMNSLRAEDTAVYYCAKSHAFDVWGQGTMVTVSS

SEQ ID NO: 113 - protein, 115 aa, synthetic construct
EVQLLESGGGLVQPGGSLRLSCAGSGFSFGSQTMSWVRQAPGKGLEWVSSISYISGRTYYADSVKGRFTISRDNSKNTLYLQMNSLRAEDTAVYYCTRSHAFDVWGQGTMVTVSS

SEQ ID NO: 114 - protein, 115 aa, synthetic construct
EVQLLESGGGLVQPGGSLRLSCAGSGFSFGSQTMSWVRQAPGKGLEWVSSISVISGRSYYADSVKGRFTISRDNSKNTLYLQMNSLRAEDTAVYYCTRSHAFDVWGQGTMVTVSS

SEQ ID NO: 115 - protein, 115 aa, synthetic construct
EVQLLESGGGLVQPGGSLRLSCAGSGFSFGSQTMSWVRQAPGKGLEWVSSISVISGRTYYADSVKGRFTISRDNSKNTLYLQMNSLRAEDTAVYYCTKQHAFDVWGQGTMVTVSS

SEQ ID NO: 116 - protein, 115 aa, synthetic construct
EVQLLESGGGLVQPGGSLRLSCAGSGFSFGSQTMSWVRQAPGKGLEWVSSISVISGRTYYADSVKGRFTISRDNSKNTLYLQMNSLRAEDTAVYYCAKSHAFDVWGQGTMVTVSS

SEQ ID NO: 117 - protein, 115 aa, synthetic construct
EVQLLESGGGLVQPGGSLRLSCAGSGFSFGSQTMSWVRQAPGKGLEWVSSISVISGRNYYADSVKGRFTISRDNSKNTLYLQMNSLRAEDTAVYYCAKSHAFDVWGQGTMVTVSS

SEQ ID NO: 118 - protein, 115 aa, synthetic construct
EVQLLESGGGLVQPGGSLRLSCAGSGFSFGSQTMSWVRQAPGKGLEWVSSISVISGRKYYADSVKGRFTISRDNSKNTLYLQMNSLRAEDTAVYYCTKSHAFDVWGQGTMVTVSS

SEQ ID NO: 119 - protein, 115 aa, synthetic construct
EVQLLESGGGLVQPGGSLRLSCAGSGFSFGSQTMSWVRQAPGKGLEWVSSISVISGRDYYADSVKGRFTISRDNSKNTLYLQMNSLRAEDTAVYYCAKSHAFDVWGQGTMVTVSS

SEQ ID NO: 120 - protein, 115 aa, synthetic construct
EVQLLESGGGLVQPGGSLRLSCAGSGFSFGSQTMSWVRQAPGKGLEWVSSISVISKRTYYADSVKGRFTISRDNSKNTLYLQMNSLRAEDTAVYYCTKSHAFDVWGQGTMVTVSS

SEQ ID NO: 121 - protein, 115 aa, synthetic construct
EVQLLESGGGLVQPGGSLRLSCAGSGFSFGSQTMSWVRQAPGKGLEWVSSISVISRRTYYADSVKGRFTISRDNSKNTLYLQMNSLRAEDTAVYYCAKSHAFDVWGQGTMVTVSS

SEQ ID NO: 122 - protein, 115 aa, synthetic construct
EVQLLESGGGLVQPGGSLRLSCAGSGFSFGSQTMSWVRQAPGKGLEWVSSISHISGRTYYADSVKGRFTISRDNSKNTLYLQMNSLRAEDTAVYYCTKSHDFDVWGQGTMVTVSS

SEQ ID NO: 123 - protein, 115 aa, synthetic construct
EVQLLESGGGLVQPGGSLRLSCAGSGFSFGSQTMSWVRQAPGKGLEWVSSISVISGRTYYADSVKGRFTISRDNSKNTLYLQMNSLRAEDTAVYYCTKAHAFDVWGQGTMVTVSS

SEQ ID NO: 124 - protein, 115 aa, synthetic construct
EVQLLESGGGLVQPGGSLRLSCAGSGFSFGSQTMSWVRQAPGKGLEWVSSISVISGRRYYADSVKGRFTISRDNSKNTLYLQMNSLRAEDTAVYYCAKSHAFDVWGQGTMVTVSS

SEQ ID NO: 125 - protein, 115 aa, synthetic construct
EVQLLESGGGLVQPGGSLRLSCAGSGFSLGSQTMSWVRQAPGKGLEWVSSISVISGRMYYADSVKGRFTISRDNSKNTLYLQMNSLRAEDTAVYYCTKSHAFDVWGQGTMVTVSS

SEQ ID NO: 126 - protein, 115 aa, synthetic construct
EVQLLESGGGLVQPGGSLRLSCAGSGFSFGSQTMSWVRQAPGKGLEWVSSSSVISGRTYYADSVKGRFTISRDNSKNTLYLQMNSLRAEDTAVYYCTRSHAFDVWGQGTMVTVSS

SEQ ID NO: 127 - protein, 115 aa, synthetic construct
EVQLLESGGGLVQPGGSLRLSCAGSGFSFGSQTMSWVRQAPGKGLEWVSSISVISGRDYYADSVKGRFTISRDNSKNTLYLQMNSLRAEDTAVYYCTRSHAFDVWGQGTMVTVSS

SEQ ID NO: 128 - protein, 115 aa, synthetic construct
EVQLLESGGGLVQPGGSLRLSCAGSGFSFGSQTMSWVRQAPGKGLEWVSSISVISGRAYYADSVKGRFTISRDNSKNTLYLQMNSLRAEDTAVYYCTRSHAFDVWGQGTMVTVSS

SEQ ID NO: 129 - protein, 115 aa, synthetic construct
EVQLLESGGGLVQPGGSLRLSCAGSGFSFGSQTMSWVRQAPGKGLEWVSSISVISGRRYYADSVKGRFTISRDNSKNTLYLQMNSLRAEDTAVYYCTKSHAFDVWGQGTMVTVSS

SEQ ID NO: 130 - protein, 115 aa, synthetic construct
EVQLLESGGGLVQPGGSLRLSCAGSGFSFGSQTMSWVRQAPGKGLEWVSSISVISGRNYYADSVKGRFTISRDNSKNTLYLQMNSLRAEDTAVYYCTRSHAFDVWGQGTMVTVSS

SEQ ID NO: 131 - protein, 121 aa, synthetic construct
EVQLVESGAEVKKPGASVKVSCKASGYTFTGYHIHWVRQAPGQGLEWMGWIRVNGGNTMYARKFQGRVTMTTDTSASTAYMELRNLTSEDTAVYYCARRPYCSGGTCSDSWGQGTLVTVSS

SEQ ID NO: 132 - protein, 126 aa, synthetic construct
QVQLQQSGGGLVQTGGSLRLACAGTGFTFSDYSMNWVRQAPGKGLEWVSYISNSRSRSSKYYADSVKGRFTISRDNAKNSLYLQMNSLRAEDTAVYYCARIGYCKNGVCGGAYDYWGQGTLVTVSS

SEQ ID NO: 133 - protein, 125 aa, synthetic construct
QVQLQESGPGLVKPSETLSLTCTVSGGSISSSSYYWVWIRQPPGKGLEWIGSIYHSGSTYYNPSLKSRVTISVDTSKNQFSLKLSSVTAADTAVYYCARAATSGWYLRYWYFDLWGRGTLVTVSS

SEQ ID NO: 134 - protein, 117 aa, synthetic construct
QVQLVESGGGLVQPGGSLRLSCAASRFAFSHYWMHWVRQAPGKGLEWVSGITSSGGSKYYADSVKGRFTISRDNSENTLYLQMNSLRADDTAVYYCVARGPPTHDSWGQGTLVTVSS

SEQ ID NO: 135 - protein, 120 aa, synthetic construct
QVQLQQSGPRLVKPSQTLSLTCAISGDSVSSNSADWNWIRQSPSRGLEWLGRTYYRSKWYNDYAVSVKSRITINPDTTKNQFSLQLNSVTPEDTAVYYCARGGPRPLDIWGQGTMVTVSS

SEQ ID NO: 136 - protein, 123 aa, synthetic construct
QVQLVQSRAEVKKPGESLRISCKASGYRFTSNWIGWVRQMPGKGLEWMGIIYPDDSDTRYSPSFQGQVTISADKSISTAYLEWSSLKASDTAMYYCVRQGSSTYYRVGWFDPWGQGTLVTVSS

SEQ ID NO: 137 - protein, 125 aa, synthetic construct
EVQLLESGGGLIQPGGSLRLSCAASAFTVSTNYMTWVRQAPGKGLEWVSVIYSGGSTYYADSVKGRFTISRDNSKNTLYLQMNSLRAEDTAVYYCARGRYYDGVDYGPKYGMDVWGQGTTVTVSS

SEQ ID NO: 138 - protein, 116 aa, synthetic construct
EVQLLESGGGLVQPGGSLRLSCAASGFTFSSYWMHWVRQAPGKGLVWVSRINLDGSSTGYADSVRGRFTISRDNAKSTLYLQMNSLRAEDTAVYYCARSSRGFDPWGQGTLVTVSS

SEQ ID NO: 139 - protein, 107 aa, synthetic construct
EIVLTQSPATLSVSPGERATLSCRASQSVYSNLAWYQQKPGQAPRLLIYGASTRATGIPARFSGSGSGTEFTLTISSLQSEDFAVYYCQQYNKWPLSFGGGTKVEIK

SEQ ID NO: 140 - protein, 107 aa, synthetic construct
EIVLTQSPATLSVSPGERATLSCRASQSVYSALAWYQQKPGQAPRLLIYGASTRATGIPARFSGSGSGTEFTLTISSLQSEDFAVYYCQQYHKWPLSFGGGTKVEIK

SEQ ID NO: 141 - protein, 107 aa, synthetic construct
EIVLTQSPATLSVSPGERATLSCRASQSVYSALAWYQQKPGQAPRLLIYGASTRATGIPARFSGSGSGTEFTLTISSLQSEDFAVYYCQQNNKWPLSFGGGTKVEIK

SEQ ID NO: 142 - protein, 107 aa, synthetic construct
EIVLTQSPATLSVSPGERATLSCRASQSVWSNLAWYQQKPGQAPRLLIYGASTRATGIPARFSGSGSGTEFTLTISSLQSEDFAVYYCQQYHKWPLSFGGGTKVEIK

SEQ ID NO: 143 - protein, 107 aa, synthetic construct
EIVLTQSPATLSVSPGERATLSCRASQSVYYNLAWYQQKPGQAPRLLIYGASTRATGIPARFSGSGSGTEFTLTISSLQSEDFAVYYCQQYHKWPLSFGGGTKVEIK

SEQ ID NO: 144 - protein, 107 aa, synthetic construct
EIVLTQSPATLSVSPGERATLSCRASQSLYSHLAWYQQKPGQAPRLLIYGASTRATGIPARFSGSGSGTEFTLTISSLQSEDFAVYYCQQYKKWPLSFGGGTKVEIK

SEQ ID NO: 145 - protein, 107 aa, synthetic construct
EIVLTQSPATLSVSPGERATLSCRASQSVYSNLAWYQQKPGQAPRLLIYGASTRATGIPARFSGSGSGTEFTLTISSLQSEDFAVYYCQQYHKWPLSFGGGTKVEIK

SEQ ID NO: 146 - protein, 107 aa, synthetic construct
EIVLTQSPATLSVSPGERATLSCRASQSVFSNLAWYQQKPGQAPRLLIYGASTRATGIPARFSGSGSGTEFTLTISSLQSEDFAVYYCQQYHWWPLSFGGGTKVEIK

SEQ ID NO: 147 - protein, 107 aa, synthetic construct
EIVLTQSPATLSVSPGERATLSCRASQSVYSALAWYQQKPGQAPRLLIYGASTRATGIPARFSGSGSGTEFTLTISSLQSEDFAVYYCQQNNRWPLSFGGGTKVEIK

SEQ ID NO: 148 - protein, 107 aa, synthetic construct
EIVLTQSPATLSVSPGERATLSCRASQSVWSNLAWYQQKPGQAPRLLIYGASTRATGIPARFSGSGSGTEFTLTISSLQSEDFAVYYCQQYQKWPLSFGGGTKVEIK

SEQ ID NO: 149 - protein, 108 aa, synthetic construct
ETTLTQSPATLSVSPGERATLSCRASESVFSNLAWYQLRPGQGPRLLIYDGNKRATGIPARFSGSGSGTEFTLTISSLQSEDFGIYYCHQYNNWPPETFGQGTKLEIK

SEQ ID NO: 150 - protein, 107 aa, synthetic construct
EIVLTQSPSAMSASVGDRVTITCRASQAIRNNLAWFQQKPGKVPKRLMNTASSLESGVPSRFSGSGSGTEFTLTITSLQPEDFASYYCLQYHDSPWTFGQGTKLEIK

SEQ ID NO: 151 - protein, 107 aa, synthetic construct
DIVMTQSPSSLSASVGDRVTITCRANQNINSYLNWYQQKPGKAPELLIYAATRLQSGVPSRFSGSRSGTDFTLTISSLQPEDFATYYCQQSYSSLRTFGHGTKVDIK

SEQ ID NO: 152 - protein, 107 aa, synthetic construct
VIWMTQSPSSLSASVGDRVTITCQASQDITKYLNWYQQKPGKAPKLLIYDASILETGVPSRFSGRGSGTEFTLTINNLQPEDFATYYCQHYNSYSWTFGQGTKLEIK

SEQ ID NO: 153 - protein, 113 aa, synthetic construct
EIVLTQSPDSLAVSLGERVTINCKSSQSVLYRSKRKPNLAWYQQKPGHPPKLLVSWASTRESGVPERFTGSGSGTDFTLTISSLQAEDVAVYFCQQYYSTPLTFGGGTKVEIK

SEQ ID NO: 154 - protein, 107 aa, synthetic construct
DIQLTQSPSSLSASVGDRVTITCRASQSISSYLNWYQQKPGKAPKLLIYAASSLQSGVPSRFSGSGSGTDFTLTISSLQPEDFATYYCQQSYSTPQTFGQGTKVDIK

SEQ ID NO: 155 - protein, 107 aa, synthetic construct
DVVMTQSPGTLSVSPGERATLSCRASQSVRYNLAWYQQKPGQAPRLLMYGASIRATDIPDRFSGSGSGTDFTLTISRLEPEDFAVYYCQFYGSSPLTFGGGTKLEIK

SEQ ID NO: 156 - protein, 108 aa, synthetic construct
EIVLTQSPGSLSMSPGERATLSCRASQSISSSYLAWYQQKPGQAPRLLIYGASRRATGIPDRFSGSGSGTDFTLTISRLEPEDLAVYYCQLYGHSAYTFGQGTKVDIK

SEQ ID NO: 157 - protein, 330 aa, synthetic construct
ASTKGPSVFPLAPSSKSTSGGTAALGCLVKDYFPEPVTVSWNSGALTSGVHTFPAVLQSSGLYSLSSVVTVPSSSLGTQTYICNVNHKPSNTKVDKKVEPKSCDKTHTCPPCPAPELLGGPSVFLFPPKPKDTLMISRTPEVTCVVVDVSHEDPEVKFNWYVDGVEVHNAKTKPREEQYNSTYRVVSVLTVLHQDWLNGKEYKCKVSNKALPAPIEKTISKAKGQPREPQVYTLPPSREEMTKNQVSLTCLVKGFYPSDIAVEWESNGQPENNYKTTPPVLDSDGSFFLYSKLTVDKSRWQQGNVFSCSVMHEALHNHYTQKSLSLSPGK

SEQ ID NO: 158 - protein, 327 aa, synthetic construct
ASTKGPSVFPLAPCSRSTSESTAALGCLVKDYFPEPVTVSWNSGALTSGVHTFPAVLQSSGLYSLSSVVTVPSSSLGTKTYTCNVDHKPSNTKVDKRVESKYGPPCPSCPAPEFLGGPSVFLFPPKPKDTLMISRTPEVTCVVVDVSQEDPEVQFNWYVDGVEVHNAKTKPREEQFNSTYRVVSVLTVLHQDWLNGKEYKCKVSNKGLPSSIEKTISKAKGQPREPQVYTLPPSQEEMTKNQVSLTCLVKGFYPSDIAVEWESNGQPENNYKTTPPVLDSDGSFFLYSRLTVDKSRWQEGNVFSCSVMHEALHNHYTQKSLSLSLGK

SEQ ID NO: 159 - protein, 107 aa, synthetic construct [sequence omitted]

SEQ ID NO: 160 - protein, 106 aa, synthetic construct
GQPKAAPSVTLFPPSSEELQANKATLVCLISDFYPGAVTVAWKADSSPVKAGVETTTPSKQSNNKYAASSYLSLTPEQWKSHRSYSCQVTHEGSTVEKTVAPTECS

SEQ ID NO: 161 - protein, 615 aa, synthetic construct
MRALLLLGFLLVSLESTLSIPPWEAPKEHKYKAEEHTVVLTVTGEPCHFPFQYHRQLYHKCTHKGRPGPQPWCATTPNFDQDQRWGYCLEPKKVKDHCSKHSPCQKGGTCVNMPSGPHCLCPQHLTGNHCQKEKCFEPQLLRFFHKNEIWYRTEQAAVARCQCKGPDAHCQRLASQACRTNPCLHGGRCLEVEGHRLCHCPVGYTGAFCDVDTKASCYDGRGLSYRGLARTTLSGAPCQPWASEATYRNVTAEQARNWGLGGHAFCRNPDNDIRPWCFVLNRDRLSWEYCDLAQCQTPTQAAPPTPVSPRLHVPLMPAQPAPPKPQPTTRTPPQSQTPGALPAKREQPPSLTRNGPLSCGQRLRKSLSSMTRVVGGLVALRGAHPYIAALYWGHSFCAGSLIAPCWVLTAAHCLQDRPAPEDLTVVLGQERRNHSCEPCQTLAVRSYRLHEAFSPVSYQHDLALLRLQEDADGSCALLSPYVQPVCLPSGAARPSETTLCQVAGWGHQFEGAEEYASFLQEAQVPFLSLERCSAPDVHGSSILPGMLCAGFLEGGTDACQGDSGGPLVCEDQAAERRLTLQGIISWGSGCGDRNKPGVYTDVAYYLAWIREHTVS